European Patent Specification EP 3 159 358 B1, published October 11, 2023. Title: Tissue factor. Applicant: Genmab. The sequence listing filed with the application follows.

SEQUENCE LISTING (112 sequences)

SEQ ID NO: 1 - protein, 126 aa, Homo sapiens
EVQLVQSGAEVKKPGESLKISCKGSGYSFTSYWIGWVRQMPGKGLEWMGIIYPGDSDTRYSPSFQGQVTISADKSISTAYLQWSSLKASDTAMYYCARIHRGAGYSSSWPGAFDIWGQGTMVTVSS

SEQ ID NO: 2 - protein, 8 aa, Homo sapiens
GYSFTSYW

SEQ ID NO: 3 - protein, 8 aa, Homo sapiens
IYPGDSDT

SEQ ID NO: 4 - protein, 19 aa, Homo sapiens
ARIHRGAGYSSSWPGAFDI

SEQ ID NO: 5 - protein, 119 aa, Homo sapiens
QVQLVESGGGVVQPGRSLRLSCVASGFTVSNDGMHWVRQAPGKGLEWVALIWYDGVNKNYADSVKGRFTISRDKSKNTLYLQMNSLRAEDTAVYYCARRPGTFYGLDVWGQGTTVTVSS

SEQ ID NO: 6 - protein, 8 aa, Homo sapiens
GFTVSNDG

SEQ ID NO: 7 - protein, 8 aa, Homo sapiens
IWYDGVNK

SEQ ID NO: 8 - protein, 12 aa, Homo sapiens
ARRPGTFYGLDV

SEQ ID NO: 9 - protein, 118 aa, Homo sapiens
EVQLLESGGGLVQPGGSLRLSCAASGFTFSNYAMSWVRQAPGKGLEWVSSISGSGDYTYYTDSVKGRFTISRDNSKNTLYLQMNSLRAEDTAVYYCARSPWGYYLDSWGQGTLVTVSS

SEQ ID NO: 10 - protein, 8 aa, Homo sapiens
GFTFSNYA

SEQ ID NO: 11 - protein, 8 aa, Homo sapiens
ISGSGDYT

SEQ ID NO: 12 - protein, 11 aa, Homo sapiens
ARSPWGYYLDS

SEQ ID NO: 13 - protein, 120 aa, Homo sapiens
EVQLLESGGGLVQPGGSLRLSCAASGFTFSSYAMSWVRQAPGKGLEWVSAISGSGDSTNYADSVKGRFTISRDNSKNTLYLQMNSLRAEDTAVYYCAKDGYFLLWYFDLWGRGTLVTVSS

SEQ ID NO: 14 - protein, 8 aa, Homo sapiens
GFTFSSYA

SEQ ID NO: 15 - protein, 8 aa, Homo sapiens
ISGSGDST

SEQ ID NO: 16 - protein, 13 aa, Homo sapiens
AKDGYFLLWYFDL

SEQ ID NO: 17 - protein, 118 aa, Homo sapiens
EVQLLESGGGLVQPGGSLRLSCAASGFTFSSYGMSWVRQAPGKGLEWVSVISGSGGTTYYADSVKGRFTISRDNSKNTLYLQMNSLRAEDTAVYYCAKAPWTYYFDYWGQGTLVTVSS

SEQ ID NO: 18 - protein, 8 aa, Homo sapiens
GFTFSSYG

SEQ ID NO: 19 - protein, 8 aa, Homo sapiens
ISGSGGTT

SEQ ID NO: 20 - protein, 11 aa, Homo sapiens
AKAPWTYYFDY

SEQ ID NO: 21 - protein, 118 aa, Homo sapiens
EVQLLESGGGLVQPGGSLRLSCAASGFTFNNYAMSWVRQAPGKGLEWVSSISGSGGRTYYADSVKGRFTISRDNSKNTLFLQMNSLRAEDTAVYYCAKTPWGYYFDYWGQGTLVTVSS

SEQ ID NO: 22 - protein, 8 aa, Homo sapiens
GFTFNNYA

SEQ ID NO: 23 - protein, 8 aa, Homo sapiens
ISGSGGRT

SEQ ID NO: 24 - protein, 11 aa, Homo sapiens
AKTPWGYYFDY

SEQ ID NO: 25 - protein, 118 aa, Homo sapiens
EVQLLESGGGLVQPGGSLRLSCAASGFTFSNYAMSWVRQAPAKGLDWVSGISGSGVTTYYADSVKGRFTISRDNSKDTLYLQMNSLRAEDTAVYFCAKTPWGYYFDYWGQGILVAVSS

SEQ ID NO: 26 - protein, 8 aa, Homo sapiens
GFTFSNYA

SEQ ID NO: 27 - protein, 8 aa, Homo sapiens
ISGSGVTT

SEQ ID NO: 28 - protein, 11 aa, Homo sapiens
AKTPWGYYFDY

SEQ ID NO: 29 - protein, 118 aa, Homo sapiens
QVQLVQSGAEVKKPGSSVKVSCKAPRGTFSYYTISWVRQAPGQGLEWMGRIIPILGVANYAQKFQGRVTITADKSTSTAYMELSSLRSEDTAVYYCAREGDRRYFDYWGQGTLVTVSS

SEQ ID NO: 30 - protein, 8 aa, Homo sapiens
RGTFSYYT

SEQ ID NO: 31 - protein, 8 aa, Homo sapiens
IIPILGVA

SEQ ID NO: 32 - protein, 11 aa, Homo sapiens
AREGDRRYFDY

SEQ ID NO: 33 - protein, 120 aa, Homo sapiens
QVQLVESGGGVVQPGRSLRLSCAASGFTFSRYAMHWVRQAPGKGLEWVAVISNDGYNDYYADSVKGRFTVSRDNSKNTLYLQMNSLRAEDTAVYYCARDGQLGRGYFDYWGQGTLVTVSS

SEQ ID NO: 34 - protein, 8 aa, Homo sapiens
GFTFSRYA

SEQ ID NO: 35 - protein, 8 aa, Homo sapiens
ISNDGYND

SEQ ID NO: 36 - protein, 13 aa, Homo sapiens
ARDGQLGRGYFDY

SEQ ID NO: 37 - protein, 120 aa, Homo sapiens
QVQLVESGGGVVQPGRSLRLSCPASGFTFSIYAMHWVRQAPGKGLEWVAVVSNDGYNKYYADSVKGRFTISRDNSKDTLYLQMNSLRAEDTAVYYCARDGQLGRGYFDYWGQGTLVTVSS

SEQ ID NO: 38 - protein, 8 aa, Homo sapiens
GFTFSIYA

SEQ ID NO: 39 - protein, 8 aa, Homo sapiens
VSNDGYNK

SEQ ID NO: 40 - protein, 13 aa, Homo sapiens
ARDGQLGRGYFDY

SEQ ID NO: 41 - protein, 118 aa, Homo sapiens
QVQLVESGGGVVQPGRSLRLSCAASGFTFSDYAMHWVRQAPGKGLEWVAVIPYDGDNKYYADSVKGRFTISRDNSKNTLYLQMNSLRAEDTAVYYCAREDWGLEVDYWGQGALVTVSS

SEQ ID NO: 42 - protein, 8 aa, Homo sapiens
GFTFSDYA

SEQ ID NO: 43 - protein, 8 aa, Homo sapiens
IPYDGDNK

SEQ ID NO: 44 - protein, 11 aa, Homo sapiens
AREDWGLEVDY

SEQ ID NO: 45 - protein, 121 aa, Homo sapiens
EVQLVQSGAEVKKPGESLKISCKGSGYSFTSCWIGWVRQMPGKGLEWMGIIYPGDSDTRYSPSFQGQVTISADKSISTAYLQWSSLKASDTAMYYCARHKLGMDHDAFDIWGQGTMVTVSS

SEQ ID NO: 46 - protein, 8 aa, Homo sapiens
GYSFTSCW

SEQ ID NO: 47 - protein, 8 aa, Homo sapiens
IYPGDSDT

SEQ ID NO: 48 - protein, 14 aa, Homo sapiens
ARHKLGMDHDAFDI

SEQ ID NO: 49 - protein, 118 aa, Homo sapiens
QVQLVQSGAEVRKPGSSVKVSCKASGGSFNNYPIFWVRQAPGQGFEWMGRIIPILGITAYAQKFQGRVTITADKSTSTAYMELNSLRSEDTAVYYCAGGDDLDAFDIWGQGTMVSVSS

SEQ ID NO: 50 - protein, 8 aa, Homo sapiens
GGSFNNYP

SEQ ID NO: 51 - protein, 8 aa, Homo sapiens
IIPILGIT

SEQ ID NO: 52 - protein, 11 aa, Homo sapiens
AGGDDLDAFDI

SEQ ID NO: 53 - protein, 120 aa, Homo sapiens
QVQLVESGGGVVQPGRSLRLSCAGSGFTFNRYAMYWVRQAPGKGLDWVAVISNDGINKYYADSVKGRFTISRDNSKNTLYLQMNSLRAEDTAVYYCARDHTMVRGAFDYWGQGTLVTVSS

SEQ ID NO: 54 - protein, 8 aa, Homo sapiens
GFTFNRYA

SEQ ID NO: 55 - protein, 8 aa, Homo sapiens
ISNDGINK

SEQ ID NO: 56 - protein, 13 aa, Homo sapiens
ARDHTMVRGAFDY

SEQ ID NO: 57 - protein, 107 aa, Homo sapiens
DIQMTQSPSSLSASVGDRVTITCRASQGISRWLAWYQQKPEKAPKSLIYAASSLQSGVPSRFSGSGSGTDFTLTISSLQPEDFATYYCQQYDSDPITFGQGTRLEIK

SEQ ID NO: 58 - protein, 6 aa, Homo sapiens
QGISRW

SEQ ID NO: 59 - protein, 3 aa, Homo sapiens
AAS

SEQ ID NO: 60 - protein, 9 aa, Homo sapiens
QQYDSDPIT

SEQ ID NO: 61 - protein, 107 aa, Homo sapiens
EIVLTQSPGTLSLSPGERATLSCRASQSVSSSYLAWYQQKPGQAPRLLIYGASSRATGIPDRFSGSGSGTDFTLTISRLEPEDFAVYYCQQYGSSLTFGGGTKVEIK

SEQ ID NO: 62 - protein, 7 aa, Homo sapiens
QSVSSSY

SEQ ID NO: 63 - protein, 3 aa, Homo sapiens
GAS

SEQ ID NO: 64 - protein, 8 aa, Homo sapiens
QQYGSSLT

SEQ ID NO: 65 - protein, 107 aa, Homo sapiens
DIQMTQSPPSLSASAGDRVTITCRASQGISSRLAWYQQKPEKAPKSLIYAASSLQSGVPSRFSGSGSGTDFTLTISSLQPEDFATYYCQQYNSYPYTFGQGTKLEIK

SEQ ID NO: 66 - protein, 6 aa, Homo sapiens
QGISSR

SEQ ID NO: 67 - protein, 3 aa, Homo sapiens
AAS

SEQ ID NO: 68 - protein, 9 aa, Homo sapiens
QQYNSYPYT

SEQ ID NO: 69 - protein, 108 aa, Homo sapiens
EIVLTQSPGTLSLSPGERATLSCRASQSVRSSYLAWYQQKPGQAPRLLIYGASSRATGIPDRFSGSGSGTDFTLTISRLEPEDFAVYYCQQYGSSPRTFGQGTKVEIK

SEQ ID NO: 70 - protein, 7 aa, Homo sapiens
QSVRSSY

SEQ ID NO: 71 - protein, 3 aa, Homo sapiens
GAS

SEQ ID NO: 72 - protein, 9 aa, Homo sapiens
QQYGSSPRT

SEQ ID NO: 73 - protein, 108 aa, Homo sapiens
EIVLTQSPGTLSLSPGERATLSCRASQSVGSSSLAWYQQKPGQAPRLLIYGASSRATGIPDRFSGSGSGTDFTLTISRLEPEDFAVYYCQQYGSSPRTFGQGTKVEIK

SEQ ID NO: 74 - protein, 7 aa, Homo sapiens
QSVGSSS

SEQ ID NO: 75 - protein, 3 aa, Homo sapiens
GAS

SEQ ID NO: 76 - protein, 9 aa, Homo sapiens
QQYGSSPRT

SEQ ID NO: 77 - protein, 107 aa, Homo sapiens
DIQMTQSPSSLSASVGDRVTITCRASQGISSRLAWYQQKPEKAPKSLIYAASSLQSGVPSRFSGSGSGTDFTLTISSLQPEDFATYYCQQYNSYPYTFGQGTKLEIK

SEQ ID NO: 78 - protein, 6 aa, Homo sapiens
QGISSR

SEQ ID NO: 79 - protein, 3 aa, Homo sapiens
AAS

SEQ ID NO: 80 - protein, 9 aa, Homo sapiens
QQYNSYPYT

SEQ ID NO: 81 - protein, 108 aa, Homo sapiens
DIQMTQSPSSLSASVGDRVTITCRASQGISSWLAWYQQKPEKAPKSLIYAASSLQSGVPSRFSGSGSGTDFTLTISSLQPEDFATYYCQQYNSYPLYTFGQGTKLEIK

SEQ ID NO: 82 - protein, 6 aa, Homo sapiens
QGISSW

SEQ ID NO: 83 - protein, 3 aa, Homo sapiens
AAS

SEQ ID NO: 84 - protein, 10 aa, Homo sapiens
QQYNSYPLYT

SEQ ID NO: 85 - protein, 107 aa, Homo sapiens
AIQLTQSPSSLSASVGDRVTITCRASQDISSALAWYQQKPGKAPKLLIYDASILESGVPSRFSGSGSGTDFTLTISSLQPEDFATYYCQQFNSYPLTFGGGTKVEIK

SEQ ID NO: 86 - protein, 6 aa, Homo sapiens
QDISSA

SEQ ID NO: 87 - protein, 3 aa, Homo sapiens
DAS

SEQ ID NO: 88 - protein, 9 aa, Homo sapiens
QQFNSYPLT

SEQ ID NO: 89 - protein, 107 aa, Homo sapiens
EIVLTQSPATLSLSPGERATLSCRASQSVSSYLAWYQQKPGQAPRLLIYDASNRATGIPARFSGSGSGTDFTLTISSLEPEDFAVYYCQQRSNWPLTFGGGTKVEIK

SEQ ID NO: 90 - protein, 6 aa, Homo sapiens
QSVSSY

SEQ ID NO: 91 - protein, 3 aa, Homo sapiens
DAS

SEQ ID NO: 92 - protein, 9 aa, Homo sapiens
QQRSNWPLT

SEQ ID NO: 93 - protein, 107 aa, Homo sapiens
EIVLTQSPATLSLSPGERAILSCRASQSVSSYLAWYQQKPGQAPRLLIYDASNRATGIPARFSGSGSGTDFTLTISSLEPEDFAVYYCQQRSNWPLTFGGGTKVEIK

SEQ ID NO: 94 - protein, 6 aa, Homo sapiens
QSVSSY

SEQ ID NO: 95 - protein, 3 aa, Homo sapiens
DAS

SEQ ID NO: 96 - protein, 9 aa, Homo sapiens
QQRSNWPLT

SEQ ID NO: 97 - protein, 107 aa, Homo sapiens
AIQLTQSPSSLSASVGDRVTITCRASQGINSALAWYQQKPGKAPKLLIYDASSLESGVPSRFSGSGSGTDFTLTISSLQPEDFATYYCQQFNSYPLTFGGGTKVEIK

SEQ ID NO: 98 - protein, 6 aa, Homo sapiens
QGINSA

SEQ ID NO: 99 - protein, 3 aa, Homo sapiens
DAS

SEQ ID NO: 100 - protein, 9 aa, Homo sapiens
QQFNSYPLT

SEQ ID NO: 101 - protein, 107 aa, Homo sapiens
DIQMTQSPSSLSASVGDRVTITCRASQGISSWLAWYQQKPEKAPKSLIYAASSLQSGVPSRFSGSGSGTDFTLTISSLQPEDFATYYCQQYNSYPPTFGQGTTVEVK

SEQ ID NO: 102 - protein, 6 aa, Homo sapiens
QGISSW

SEQ ID NO: 103 - protein, 3 aa, Homo sapiens
AAS

SEQ ID NO: 104 - protein, 9 aa, Homo sapiens
QQYNSYPPT

SEQ ID NO: 105 - protein, 107 aa, Homo sapiens
DIQMTQSPSSLSASVGDRVTITCRASQGISSWLAWYQQKPEKAPKSLIYAASSLQSGVPSRFSGSGSGTDFTLTISSLQPEDFATYYCQQYNSYPYTFGQGTKLEIK

SEQ ID NO: 106 - protein, 6 aa, Homo sapiens
QGISSW

SEQ ID NO: 107 - protein, 3 aa, Homo sapiens
AAS

SEQ ID NO: 108 - protein, 9 aa, Homo sapiens
QQYNSYPYT

SEQ ID NO: 109 - protein, 107 aa, Homo sapiens; identical to SEQ ID NO: 89

SEQ ID NO: 110 - protein, 6 aa, Homo sapiens
QSVSSY

SEQ ID NO: 111 - protein, 3 aa, Homo sapiens
DAS

SEQ ID NO: 112 - protein, 9 aa, Homo sapiens
QQRSNWPLT